European Patent Application EP 4 768 038 A1, published July 1, 2026. Title: Novel use of a nonapeptide. Applicant: ENSOL BIOSCIENCES INC. Application KR. The sequence listing filed with the application follows.

SEQUENCE LISTING (1 sequence)

SEQ ID NO: 1 - protein, 9 aa, synthetic construct
YGAGAGAGY